European Patent Application EP 4 497 756 A2, published January 29, 2025. Title: 检测促甲状腺激素的抗体、试剂盒、检测方法、以及样本分析仪. Applicant: 深圳迈瑞生物医疗电子股份有限公司. Application CN. The sequence listing filed with the application follows.

SEQUENCE LISTING (206 sequences)

SEQ ID NO: 1 - protein, 7 aa, synthetic construct
  source 1..7: note = Amino acid sequence of CDR-H1 of TS01/rTS01
TYYYYMC

SEQ ID NO: 2 - protein, 18 aa, synthetic construct
  source 1..18: note = Amino acid sequence of CDR-H2 of TS01/rTS01
CIEAGGSGTTYYANWAKG

SEQ ID NO: 3 - protein, 17 aa, synthetic construct
  source 1..17: note = Amino acid sequence of CDR-H3 of TS01/rTS01
FLGYASDGGAYINAFNL

SEQ ID NO: 4 - protein, 11 aa, synthetic construct
  source 1..11: note = Amino acid sequence of CDR-L1 of TS01/rTS01
QASQNIGSNLA

SEQ ID NO: 5 - protein, 7 aa, synthetic construct
  source 1..7: note = Amino acid sequence of CDR-L2 of TS01/rTS01
RASTLES

SEQ ID NO: 6 - protein, 12 aa, synthetic construct
  source 1..12: note = Amino acid sequence of CDR-L3 of TS01/rTS01
QCTVYGSSDVFA

SEQ ID NO: 7 - protein, 5 aa, synthetic construct
  source 1..5: note = Amino acid sequence of CDR-H1 of TS02/rTS02
SNAVG

SEQ ID NO: 8 - protein, 16 aa, synthetic construct
  source 1..16: note = Amino acid sequence of CDR-H2 of TS02/rTS02
GMSSGGSTYYNPALKS

SEQ ID NO: 9 - protein, 14 aa, synthetic construct
  source 1..14: note = Amino acid sequence of CDR-H3 of TS02/rTS02
VDATRPDDIGWIDY

SEQ ID NO: 10 - protein, 11 aa, synthetic construct
  source 1..11: note = Amino acid sequence of CDR-L1 of TS02/rTS02
SGSDIGSSAVG

SEQ ID NO: 11 - protein, 7 aa, synthetic construct
  source 1..7: note = Amino acid sequence of CDR-L2 of TS02/rTS02
GTVRRPS

SEQ ID NO: 12 - protein, 10 aa, synthetic construct
  source 1..10: note = Amino acid sequence of CDR-L3 of TS02/rTS02
GGAAGSNYGD

SEQ ID NO: 13 - protein, 5 aa, synthetic construct
  source 1..5: note = Amino acid sequence of CDR-H1 of TS03/rTS03
SNAVG

SEQ ID NO: 14 - protein, 16 aa, synthetic construct
  source 1..16: note = Amino acid sequence of CDR-H2 of TS03/rTS03
GISSGGTAYYNPALKS

SEQ ID NO: 15 - protein, 14 aa, synthetic construct
  source 1..14: note = Amino acid sequence of CDR-H3 of TS03/rTS03
VDATRPDDIGWIDY

SEQ ID NO: 16 - protein, 11 aa, synthetic construct
  source 1..11: note = Amino acid sequence of CDR-L1 of TS03/rTS03
SGSDFGSSAVG

SEQ ID NO: 17 - protein, 7 aa, synthetic construct
  source 1..7: note = Amino acid sequence of CDR-L2 of TS03/rTS03
GTTRRPS

SEQ ID NO: 18 - protein, 10 aa, synthetic construct
  source 1..10: note = Amino acid sequence of CDR-L3 of TS03/rTS03
GGAAGSDHGD

SEQ ID NO: 19 - protein, 5 aa, synthetic construct
  source 1..5: note = Amino acid sequence of CDR-H1 of TS04/rTS04
NYDVG

SEQ ID NO: 20 - protein, 16 aa, synthetic construct
  source 1..16: note = Amino acid sequence of CDR-H2 of TS04/rTS04
DIYSGGGKSYNPALKS

SEQ ID NO: 21 - protein, 14 aa, synthetic construct
  source 1..14: note = Amino acid sequence of CDR-H3 of TS04/rTS04
GVYSGNGIADAADV

SEQ ID NO: 22 - protein, 11 aa, synthetic construct
  source 1..11: note = Amino acid sequence of CDR-L1 of TS04/rTS04
SGSYIDSRHVG

SEQ ID NO: 23 - protein, 6 aa, synthetic construct
  source 1..6: note = Amino acid sequence of CDR-L2 of TS04/rTS04
YSTNRP

SEQ ID NO: 24 - protein, 11 aa, synthetic construct
  source 1..11: note = Amino acid sequence of CDR-L3 of TS04/rTS04
GSYAASIDEGI

SEQ ID NO: 25 - protein, 5 aa, synthetic construct
  source 1..5: note = Amino acid sequence of CDR-H1 of TS05/rTS05
MYSIT

SEQ ID NO: 26 - protein, 16 aa, synthetic construct
  source 1..16: note = Amino acid sequence of CDR-H2 of TS05/rTS05
DIWGDGSTLYNPALKS

SEQ ID NO: 27 - protein, 11 aa, synthetic construct
  source 1..11: note = Amino acid sequence of CDR-H3 of TS05/rTS05
GVGTTVTEVDD

SEQ ID NO: 28 - protein, 11 aa, synthetic construct
  source 1..11: note = Amino acid sequence of CDR-L1 of TS05/rTS05
QGDLLDDQYTA

SEQ ID NO: 29 - protein, 7 aa, synthetic construct
  source 1..7: note = Amino acid sequence of CDR-L2 of TS05/rTS05
KDTERPS

SEQ ID NO: 30 - protein, 10 aa, synthetic construct
  source 1..10: note = Amino acid sequence of CDR-L3 of TS05/rTS05
LSLDSSRMGV

SEQ ID NO: 31 - protein, 5 aa, synthetic construct
  source 1..5: note = Amino acid sequence of CDR-H1 of TS06/rTS06
SNAVG

SEQ ID NO: 32 - protein, 16 aa, synthetic construct
  source 1..16: note = Amino acid sequence of CDR-H2 of TS06/rTS06
GISSGGSAYYNPALKS

SEQ ID NO: 33 - protein, 14 aa, synthetic construct
  source 1..14: note = Amino acid sequence of CDR-H3 of TS06/rTS06
VDATRPDDIGWVDF

SEQ ID NO: 34 - protein, 11 aa, synthetic construct
  source 1..11: note = Amino acid sequence of CDR-L1 of TS06/rTS06
SGSDFFSNAVG

SEQ ID NO: 35 - protein, 7 aa, synthetic construct
  source 1..7: note = Amino acid sequence of CDR-L2 of TS06/rTS06
GTTRRPS

SEQ ID NO: 36 - protein, 10 aa, synthetic construct
  source 1..10: note = Amino acid sequence of CDR-L3 of TS06/rTS06
GSTARSNYGD

SEQ ID NO: 37 - protein, 5 aa, synthetic construct
  source 1..5: note = Amino acid sequence of CDR-H1 of TS07/rTS07
SNAVG

SEQ ID NO: 38 - protein, 16 aa, synthetic construct
  source 1..16: note = Amino acid sequence of CDR-H2 of TS07/rTS07
GISSGGTTYYNPALKS

SEQ ID NO: 39 - protein, 14 aa, synthetic construct
  source 1..14: note = Amino acid sequence of CDR-H3 of TS07/rTS07
VDATRPDDIGWIDY

SEQ ID NO: 40 - protein, 11 aa, synthetic construct
  source 1..11: note = Amino acid sequence of CDR-L1 of TS07/rTS07
SGSDFGSSAVG

SEQ ID NO: 41 - protein, 7 aa, synthetic construct
  source 1..7: note = Amino acid sequence of CDR-L2 of TS07/rTS07
GTTRRPS

SEQ ID NO: 42 - protein, 10 aa, synthetic construct
  source 1..10: note = Amino acid sequence of CDR-L3 of TS07/rTS07
GGAAGTNHGD

SEQ ID NO: 43 - protein, 5 aa, synthetic construct
  source 1..5: note = Amino acid sequence of CDR-H1 of TS08/rTS08
SYSVN

SEQ ID NO: 44 - protein, 16 aa, synthetic construct
  source 1..16: note = Amino acid sequence of CDR-H2 of TS08/rTS08
DISTYGNTVYNPTLES

SEQ ID NO: 45 - protein, 15 aa, synthetic construct
  source 1..15: note = Amino acid sequence of CDR-H3 of TS08/rTS08
LHLTDSSHTRNGVDV

SEQ ID NO: 46 - protein, 10 aa, synthetic construct
  source 1..10: note = Amino acid sequence of CDR-L1 of TS08/rTS08
QGDIGSSYVA

SEQ ID NO: 47 - protein, 7 aa, synthetic construct
  source 1..7: note = Amino acid sequence of CDR-L2 of TS08/rTS08
QNSKRPS

SEQ ID NO: 48 - protein, 8 aa, synthetic construct
  source 1..8: note = Amino acid sequence of CDR-L3 of TS08/rTS08
LSADSRFV

SEQ ID NO: 49 - protein, 5 aa, synthetic construct
  source 1..5: note = Amino acid sequence of CDR-H1 of TS09/rTS09
SYNVV

SEQ ID NO: 50 - protein, 16 aa, synthetic construct
  source 1..16: note = Amino acid sequence of CDR-H2 of TS09/rTS09
EIEPGGSTFSNPALKS

SEQ ID NO: 51 - protein, 8 aa, synthetic construct
  source 1..8: note = Amino acid sequence of CDR-H3 of TS09/rTS09
ASYTDALR

SEQ ID NO: 52 - protein, 14 aa, synthetic construct
  source 1..14: note = Amino acid sequence of CDR-L1 of TS09/rTS09
SGSSSNIGGGYYVG

SEQ ID NO: 53 - protein, 7 aa, synthetic construct
  source 1..7: note = Amino acid sequence of CDR-L2 of TS09/rTS09
QNSKRPT

SEQ ID NO: 54 - protein, 11 aa, synthetic construct
  source 1..11: note = Amino acid sequence of CDR-L3 of TS09/rTS09
STYDSSISASV

SEQ ID NO: 55 - protein, 5 aa, synthetic construct
  source 1..5: note = Amino acid sequence of CDR-H1 of TS10/rTS10
SYSVN

SEQ ID NO: 56 - protein, 16 aa, synthetic construct
  source 1..16: note = Amino acid sequence of CDR-H2 of TS10/rTS10
DISTYGNTVYNPALES

SEQ ID NO: 57 - protein, 15 aa, synthetic construct
  source 1..15: note = Amino acid sequence of CDR-H3 of TS10/rTS10
LRLSEGGHTRNGVDV

SEQ ID NO: 58 - protein, 11 aa, synthetic construct
  source 1..11: note = Amino acid sequence of CDR-L1 of TS10/rTS10
QGDDIGRSYVA

SEQ ID NO: 59 - protein, 7 aa, synthetic construct
  source 1..7: note = Amino acid sequence of CDR-L2 of TS10/rTS10
QNSKRPS

SEQ ID NO: 60 - protein, 8 aa, synthetic construct
  source 1..8: note = Amino acid sequence of CDR-L3 of TS10/rTS10
LSAGSRFV

SEQ ID NO: 61 - protein, 5 aa, synthetic construct
  source 1..5: note = Amino acid sequence of CDR-H1 of TS11/rTS11
SNAVH

SEQ ID NO: 62 - protein, 16 aa, synthetic construct
  source 1..16: note = Amino acid sequence of CDR-H2 of TS11/rTS11
VIVSTGSTAYNPALKS

SEQ ID NO: 63 - protein, 16 aa, synthetic construct
  source 1..16: note = Amino acid sequence of CDR-H3 of TS11/rTS11
TIGGDDWTSDVEHIDY

SEQ ID NO: 64 - protein, 13 aa, synthetic construct
  source 1..13: note = Amino acid sequence of CDR-L1 of TS11/rTS11
SGSSRNVGEYGVG

SEQ ID NO: 65 - protein, 7 aa, synthetic construct
  source 1..7: note = Amino acid sequence of CDR-L2 of TS11/rTS11
GTSSRPS

SEQ ID NO: 66 - protein, 11 aa, synthetic construct
  source 1..11: note = Amino acid sequence of CDR-L3 of TS11/rTS11
ATTDSSRRNVV

SEQ ID NO: 67 - protein, 5 aa, synthetic construct
  source 1..5: note = Amino acid sequence of CDR-H1 of TS12/rTS12
SDAVT

SEQ ID NO: 68 - protein, 16 aa, synthetic construct
  source 1..16: note = Amino acid sequence of CDR-H2 of TS12/rTS12
IIYSGGSTSYNQTLKS

SEQ ID NO: 69 - protein, 11 aa, synthetic construct
  source 1..11: note = Amino acid sequence of CDR-H3 of TS12/rTS12
SNFGYDSDLDY

SEQ ID NO: 70 - protein, 14 aa, synthetic construct
  source 1..14: note = Amino acid sequence of CDR-L1 of TS12/rTS12
SGSSSNVGYGNYVG

SEQ ID NO: 71 - protein, 7 aa, synthetic construct
  source 1..7: note = Amino acid sequence of CDR-L2 of TS12/rTS12
GATNRAS

SEQ ID NO: 72 - protein, 10 aa, synthetic construct
  source 1..10: note = Amino acid sequence of CDR-L3 of TS12/rTS12
ASYDSSSRIV

SEQ ID NO: 73 - protein, 5 aa, synthetic construct
  source 1..5: note = Amino acid sequence of CDR-H1 of TS13/rTS13
TKAVH

SEQ ID NO: 74 - protein, 16 aa, synthetic construct
  source 1..16: note = Amino acid sequence of CDR-H2 of TS13/rTS13
VIASSGSTAYNPALKS

SEQ ID NO: 75 - protein, 16 aa, synthetic construct
  source 1..16: note = Amino acid sequence of CDR-H3 of TS13/rTS13
TIGGDDWRSDVEHIDY

SEQ ID NO: 76 - protein, 13 aa, synthetic construct
  source 1..13: note = Amino acid sequence of CDR-L1 of TS13/rTS13
SGSSRNVGEYGVA

SEQ ID NO: 77 - protein, 7 aa, synthetic construct
  source 1..7: note = Amino acid sequence of CDR-L2 of TS13/rTS13
GTSNRPS

SEQ ID NO: 78 - protein, 11 aa, synthetic construct
  source 1..11: note = Amino acid sequence of CDR-L3 of TS13/rTS13
AATDSSRRDVV

SEQ ID NO: 79 - protein, 5 aa, synthetic construct
  source 1..5: note = Amino acid sequence of CDR-H1 of TS14/rTS14
SYNLV

SEQ ID NO: 80 - protein, 16 aa, synthetic construct
  source 1..16: note = Amino acid sequence of CDR-H2 of TS14/rTS14
EIEPGGSTFYNPALKS

SEQ ID NO: 81 - protein, 8 aa, synthetic construct
  source 1..8: note = Amino acid sequence of CDR-H3 of TS14/rTS14
ASHTDFLR

SEQ ID NO: 82 - protein, 14 aa, synthetic construct
  source 1..14: note = Amino acid sequence of CDR-L1 of TS14/rTS14
SGSSSNIGGGYYVG

SEQ ID NO: 83 - protein, 7 aa, synthetic construct
  source 1..7: note = Amino acid sequence of CDR-L2 of TS14/rTS14
QNSKRPT

SEQ ID NO: 84 - protein, 11 aa, synthetic construct
  source 1..11: note = Amino acid sequence of CDR-L3 of TS14/rTS14
STYDSSISTTV

SEQ ID NO: 85 - protein, 5 aa, synthetic construct
  source 1..5: note = Amino acid sequence of CDR-H1 of TS15/rTS15
SNAVH

SEQ ID NO: 86 - protein, 16 aa, synthetic construct
  source 1..16: note = Amino acid sequence of CDR-H2 of TS15/rTS15
GIVSSGSTAYNPALKS

SEQ ID NO: 87 - protein, 16 aa, synthetic construct
  source 1..16: note = Amino acid sequence of CDR-H3 of TS15/rTS15
TIGGDDWTSNVEHIDY

SEQ ID NO: 88 - protein, 13 aa, synthetic construct
  source 1..13: note = Amino acid sequence of CDR-L1 of TS15/rTS15
SGSSRNVGEYGVG

SEQ ID NO: 89 - protein, 7 aa, synthetic construct
  source 1..7: note = Amino acid sequence of CDR-L2 of TS15/rTS15
GTRSRPS

SEQ ID NO: 90 - protein, 11 aa, synthetic construct
  source 1..11: note = Amino acid sequence of CDR-L3 of TS15/rTS15
ATTDSSRRNVV

SEQ ID NO: 91 - protein, 5 aa, synthetic construct
  source 1..5: note = Amino acid sequence of CDR-H1 of TS16/rTS16
TYAVT

SEQ ID NO: 92 - protein, 16 aa, synthetic construct
  source 1..16: note = Amino acid sequence of CDR-H2 of TS16/rTS16
IIYSGGSTSYNQTLKS

SEQ ID NO: 93 - protein, 11 aa, synthetic construct
  source 1..11: note = Amino acid sequence of CDR-H3 of TS16/rTS16
SNFGYDSDLDY

SEQ ID NO: 94 - protein, 14 aa, synthetic construct
  source 1..14: note = Amino acid sequence of CDR-L1 of TS16/rTS16
SGSSSNVGYGNYVG

SEQ ID NO: 95 - protein, 7 aa, synthetic construct
  source 1..7: note = Amino acid sequence of CDR-L2 of TS16/rTS16
GATNRAS

SEQ ID NO: 96 - protein, 10 aa, synthetic construct
  source 1..10: note = Amino acid sequence of CDR-L3 of TS16/rTS16
ASYDINSRII

SEQ ID NO: 97 - protein, 5 aa, synthetic construct
  source 1..5: note = Amino acid sequence of CDR-H1 of TS17/rTS17
NDGVG

SEQ ID NO: 98 - protein, 16 aa, synthetic construct
  source 1..16: note = Amino acid sequence of CDR-H2 of TS17/rTS17
AIYSSGGTYYNPALKS

SEQ ID NO: 99 - protein, 17 aa, synthetic construct
  source 1..17: note = Amino acid sequence of CDR-H3 of TS17/rTS17
HFYRDWASGSDMVSFDY

SEQ ID NO: 100 - protein, 14 aa, synthetic construct
  source 1..14: note = Amino acid sequence of CDR-L1 of TS17/rTS17
SGSSGNVGFGDYVA

SEQ ID NO: 101 - protein, 7 aa, synthetic construct
  source 1..7: note = Amino acid sequence of CDR-L2 of TS17/rTS17
RATSRAS

SEQ ID NO: 102 - protein, 10 aa, synthetic construct
  source 1..10: note = Amino acid sequence of CDR-L3 of TS17/rTS17
ASFDSSASGI

SEQ ID NO: 103 - protein, 92 aa, synthetic construct
  source 1..92: note = TSH alpha-subunit
APDVQDCPECTLQENPFFSQPGAPILQCMGCCFSRAYPTPLRSKKTMLVQKNVTSESTCCVAKSYNRVTVMGGFKVENHTACHCSTCYYHKS

SEQ ID NO: 104 - protein, 118 aa, synthetic construct
  source 1..118: note = TSH beta-subunit containing R55G mutation
FCIPTEYTMHIERRECAYCLTINTTICAGYCMTRDINGKLFLPKYALSQDVCTYGDFIYRTVEIPGCPLHVAPYFSYPVALSCKCGKCNTDYSDCIHEAIKTNYCTKPQKSYLVGFSV

SEQ ID NO: 105 - DNA, 21 bp, synthetic construct
  source 1..21: mol_type = other DNA; note = TS01/rTS01 CDR-H1 nucleotide sequence
acctactactactacatgtgc

SEQ ID NO: 106 - DNA, 54 bp, synthetic construct
  source 1..54: mol_type = other DNA; note = TS01/rTS01 CDR-H2 nucleotide sequence
tgtattgaggctggtggtagtggtaccacttactacgcgaactgggcgaaaggc

SEQ ID NO: 107 - DNA, 51 bp, synthetic construct
  source 1..51: mol_type = other DNA; note = TS01/rTS01 CDR-H3 nucleotide sequence
tttttgggttacgctagtgatggtggtgcttatattaacgccttcaatttg

SEQ ID NO: 108 - DNA, 15 bp, synthetic construct
  source 1..15: mol_type = other DNA; note = TS02/hTS02 CDR-H1 nucleotide sequence
agcaatgctgtaggc

SEQ ID NO: 109 - DNA, 48 bp, synthetic construct
  source 1..48: mol_type = other DNA; note = TS02/hTS02 CDR-H2 nucleotide sequence
ggcatgagtagtggtggaagtacatactataacccggccctgaaatcc

SEQ ID NO: 110 - DNA, 42 bp, synthetic construct
  source 1..42: mol_type = other DNA; note = TS02/hTS02 CDR-H3 nucleotide sequence
gttgatgcgactcgtcctgatgatattggttggatcgactac

SEQ ID NO: 111 - DNA, 15 bp, synthetic construct
  source 1..15: mol_type = other DNA; note = TS03/hTS03 CDR-H1 nucleotide sequence
agcaatgctgtcggc

SEQ ID NO: 112 - DNA, 48 bp, synthetic construct
  source 1..48: mol_type = other DNA; note = TS03/hTS03 CDR-H2 nucleotide sequence
ggcataagtagtggtggcacagcatactataatccggccctgaaatcc

SEQ ID NO: 113 - DNA, 42 bp, synthetic construct
  source 1..42: mol_type = other DNA; note = TS03/hTS03 CDR-H3 nucleotide sequence
gttgacgcgactcgtcctgatgatattggttggatcgactat

SEQ ID NO: 114 - DNA, 15 bp, synthetic construct
  source 1..15: mol_type = other DNA; note = TS04/hTS04 CDR-H1 nucleotide sequence
aattatgatgtaggc

SEQ ID NO: 115 - DNA, 48 bp, synthetic construct
  source 1..48: mol_type = other DNA; note = TS04/hTS04 CDR-H2 nucleotide sequence
gacatctatagtggtggaggtaaaagctataacccggccctgaaatcc

SEQ ID NO: 116 - DNA, 42 bp, synthetic construct
  source 1..42: mol_type = other DNA; note = TS04/hTS04 CDR-H3 nucleotide sequence
ggggtctatagtggtaatggtattgctgatgctgctgatgtc

SEQ ID NO: 117 - DNA, 15 bp, synthetic construct
  source 1..15: mol_type = other DNA; note = TS05/hTS05 CDR-H1 nucleotide sequence
atgtatagtataacc

SEQ ID NO: 118 - DNA, 48 bp, synthetic construct
  source 1..48: mol_type = other DNA; note = TS05/hTS05 CDR-H2 nucleotide sequence
gatatatggggtgatggaagtacgctctataacccggccctcaaatcc

SEQ ID NO: 119 - DNA, 33 bp, synthetic construct
  source 1..33: mol_type = other DNA; note = TS05/hTS05 CDR-H3 nucleotide sequence
ggtgttgggacgactgtgacagaagtcgacgac

SEQ ID NO: 120 - DNA, 15 bp, synthetic construct
  source 1..15: mol_type = other DNA; note = TS06/hTS06 CDR-H1 nucleotide sequence
agcaatgctgtaggc

SEQ ID NO: 121 - DNA, 48 bp, synthetic construct
  source 1..48: mol_type = other DNA; note = TS06/hTS06 CDR-H2 nucleotide sequence
ggcataagtagtggtggaagtgcatactataacccggccctgaaatcc

SEQ ID NO: 122 - DNA, 42 bp, synthetic construct
  source 1..42: mol_type = other DNA; note = TS06/hTS06 CDR-H3 nucleotide sequence
gttgatgcgactcgtcctgatgatattggttgggtcgacttc

SEQ ID NO: 123 - DNA, 15 bp, synthetic construct
  source 1..15: mol_type = other DNA; note = TS07/hTS07 CDR-H1 nucleotide sequence
agcaatgctgtcggc

SEQ ID NO: 124 - DNA, 48 bp, synthetic construct
  source 1..48: mol_type = other DNA; note = TS07/hTS07 CDR-H2 nucleotide sequence
ggcataagtagtggtggcactacatactataatccggccctgaaatcc

SEQ ID NO: 125 - DNA, 42 bp, synthetic construct
  source 1..42: mol_type = other DNA; note = TS07/hTS07 CDR-H3 nucleotide sequence
gttgatgcgactcgtcctgatgatattggttggatcgactat

SEQ ID NO: 126 - DNA, 15 bp, synthetic construct
  source 1..15: mol_type = other DNA; note = TS08/hTS08 CDR-H1 nucleotide sequence
agctatagtgtaaac

SEQ ID NO: 127 - DNA, 48 bp, synthetic construct
  source 1..48: mol_type = other DNA; note = TS08/hTS08 CDR-H2 nucleotide sequence
gatataagtacttatggaaacacagtctataacccgaccctggaatcc

SEQ ID NO: 128 - DNA, 45 bp, synthetic construct
  source 1..45: mol_type = other DNA; note = TS08/hTS08 CDR-H3 nucleotide sequence
cttcacttgactgatagtagtcatactcgaaacggtgtggatgtc

SEQ ID NO: 129 - DNA, 15 bp, synthetic construct
  source 1..15: mol_type = other DNA; note = TS09/hTS09 CDR-H1 nucleotide sequence
agctataatgtagtc

SEQ ID NO: 130 - DNA, 48 bp, synthetic construct
  source 1..48: mol_type = other DNA; note = TS09/hTS09 CDR-H2 nucleotide sequence
gaaatagaacctggtggaagtacattcagtaacccggccctgaaatcc

SEQ ID NO: 131 - DNA, 24 bp, synthetic construct
  source 1..24: mol_type = other DNA; note = TS09/hTS09 CDR-H3 nucleotide sequence
gcttcgtataccgatgcactgcga

SEQ ID NO: 132 - DNA, 15 bp, synthetic construct
  source 1..15: mol_type = other DNA; note = TS10/hTS10 CDR-H1 nucleotide sequence
agctatagtgtaaac

SEQ ID NO: 133 - DNA, 48 bp, synthetic construct
  source 1..48: mol_type = other DNA; note = TS10/hTS10 CDR-H2 nucleotide sequence
gatataagcacttatggaaacacagtctataacccggccctggaatcc

SEQ ID NO: 134 - DNA, 45 bp, synthetic construct
  source 1..45: mol_type = other DNA; note = TS10/hTS10 CDR-H3 nucleotide sequence
cttcgcttgagtgaaggtggtcacactcgaaacggtgtagatgtc

SEQ ID NO: 135 - DNA, 15 bp, synthetic construct
  source 1..15: mol_type = other DNA; note = TS11/hTS11 CDR-H1 nucleotide sequence
agcaatgctgtacac

SEQ ID NO: 136 - DNA, 48 bp, synthetic construct
  source 1..48: mol_type = other DNA; note = TS11/hTS11 CDR-H2 nucleotide sequence
gttatagttagtactgggagcacagcctataacccggccctgaaatcc

SEQ ID NO: 137 - DNA, 48 bp, synthetic construct
  source 1..48: mol_type = other DNA; note = TS11/hTS11 CDR-H3 nucleotide sequence
acaataggtggtgatgactggactagtgatgtagaacatatcgactac

SEQ ID NO: 138 - DNA, 15 bp, synthetic construct
  source 1..15: mol_type = other DNA; note = TS12/hTS12 CDR-H1 nucleotide sequence
agcgatgctgtaact

SEQ ID NO: 139 - DNA, 48 bp, synthetic construct
  source 1..48: mol_type = other DNA; note = TS12/hTS12 CDR-H2 nucleotide sequence
atcatatatagtggtggaagtacatcttataatcagaccctgaaatcc

SEQ ID NO: 140 - DNA, 33 bp, synthetic construct
  source 1..33: mol_type = other DNA; note = TS12/hTS12 CDR-H3 nucleotide sequence
agtaattttggttatgattccgatctcgactac

SEQ ID NO: 141 - DNA, 15 bp, synthetic construct
  source 1..15: mol_type = other DNA; note = TS13/hTS13 CDR-H1 nucleotide sequence
accaaggcggtacac

SEQ ID NO: 142 - DNA, 48 bp, synthetic construct
  source 1..48: mol_type = other DNA; note = TS13/hTS13 CDR-H2 nucleotide sequence
gttattgctagtagtgggagcacagcctataacccggccctgaaatcc

SEQ ID NO: 143 - DNA, 48 bp, synthetic construct
  source 1..48: mol_type = other DNA; note = TS13/hTS13 CDR-H3 nucleotide sequence
acaataggtggtgatgactggcgtagtgatgtggagcatatcgactac

SEQ ID NO: 144 - DNA, 15 bp, synthetic construct
  source 1..15: mol_type = other DNA; note = TS14/hTS14 CDR-H1 nucleotide sequence
agctataatttagtc

SEQ ID NO: 145 - DNA, 48 bp, synthetic construct
  source 1..48: mol_type = other DNA; note = TS14/hTS14 CDR-H2 nucleotide sequence
gaaatagaacctggtggaagtacattctataacccggccctgaaatcc

SEQ ID NO: 146 - DNA, 24 bp, synthetic construct
  source 1..24: mol_type = other DNA; note = TS14/hTS14 CDR-H3 nucleotide sequence
gcttcgcataccgatttcctgcga

SEQ ID NO: 147 - DNA, 15 bp, synthetic construct
  source 1..15: mol_type = other DNA; note = TS15/hTS15 CDR-H1 nucleotide sequence
agcaatgctgtacac

SEQ ID NO: 148 - DNA, 48 bp, synthetic construct
  source 1..48: mol_type = other DNA; note = TS15/hTS15 CDR-H2 nucleotide sequence
ggtatagttagtagtggaagcacagcctataacccggccctgaaatcc

SEQ ID NO: 149 - DNA, 48 bp, synthetic construct
  source 1..48: mol_type = other DNA; note = TS15/hTS15 CDR-H3 nucleotide sequence
acaataggtggtgatgactggactagtaatgtagagcatatcgactac

SEQ ID NO: 150 - DNA, 15 bp, synthetic construct
  source 1..15: mol_type = other DNA; note = TS16/hTS16 CDR-H1 nucleotide sequence
acctatgctgtaact

SEQ ID NO: 151 - DNA, 48 bp, synthetic construct
  source 1..48: mol_type = other DNA; note = TS16/hTS16 CDR-H2 nucleotide sequence
atcatatatagtggtggaagtacatcttataaccagaccctgaaatcc

SEQ ID NO: 152 - DNA, 33 bp, synthetic construct; identical to SEQ ID NO: 140
  source 1..33: mol_type = other DNA; note = TS16/hTS16 CDR-H3 nucleotide sequence

SEQ ID NO: 153 - DNA, 15 bp, synthetic construct
  source 1..15: mol_type = other DNA; note = TS17/hTS17 CDR-H1 nucleotide sequence
aacgatggtgtaggc

SEQ ID NO: 154 - DNA, 48 bp, synthetic construct
  source 1..48: mol_type = other DNA; note = TS17/hTS17 CDR-H2 nucleotide sequence
gcgatttacagtagtggaggtacatactataatccggccctgaaatcc

SEQ ID NO: 155 - DNA, 51 bp, synthetic construct
  source 1..51: mol_type = other DNA; note = TS17/hTS17 CDR-H3 nucleotide sequence
cacttttaccgtgattgggctagtgggtctgatatggtttctttcgactac

SEQ ID NO: 156 - DNA, 33 bp, synthetic construct
  source 1..33: mol_type = other DNA; note = TS01/rTS01 CDR-L1 nucleotide sequence
caggccagtcagaacattggtagtaatttagcc

SEQ ID NO: 157 - DNA, 21 bp, synthetic construct
  source 1..21: mol_type = other DNA; note = TS01/rTS01 CDR-L2 nucleotide sequence
agggcatccactctggaatct

SEQ ID NO: 158 - DNA, 36 bp, synthetic construct
  source 1..36: mol_type = other DNA; note = TS01/rTS01 CDR-L3 nucleotide sequence
caatgtactgtttatggtagtagtgatgtttttgct

SEQ ID NO: 159 - DNA, 33 bp, synthetic construct
  source 1..33: mol_type = other DNA; note = TS02/hTS02 CDR-L1 nucleotide sequence
tctggaagcgacatcggtagtagtgcagtaggc

SEQ ID NO: 160 - DNA, 21 bp, synthetic construct
  source 1..21: mol_type = other DNA; note = TS02/hTS02 CDR-L2 nucleotide sequence
ggtactgtccgtcgaccctca

SEQ ID NO: 161 - DNA, 30 bp, synthetic construct
  source 1..30: mol_type = other DNA; note = TS02/hTS02 CDR-L3 nucleotide sequence
ggaggtgctgctggtagtaactatggtgat

SEQ ID NO: 162 - DNA, 33 bp, synthetic construct
  source 1..33: mol_type = other DNA; note = TS03/hTS03 CDR-L1 nucleotide sequence
tctggaagcgacttcggtagtagtgcagtaggc

SEQ ID NO: 163 - DNA, 21 bp, synthetic construct
  source 1..21: mol_type = other DNA; note = TS03/hTS03 CDR-L2 nucleotide sequence
ggtactaccaggcgaccctca

SEQ ID NO: 164 - DNA, 30 bp, synthetic construct
  source 1..30: mol_type = other DNA; note = TS03/hTS03 CDR-L3 nucleotide sequence
ggaggtgctgctggttctgaccatggtgat

SEQ ID NO: 165 - DNA, 33 bp, synthetic construct
  source 1..33: mol_type = other DNA; note = TS04/hTS04 CDR-L1 nucleotide sequence
tctggaagctacatcgatagtaggcatgtaggc

SEQ ID NO: 166 - DNA, 21 bp, synthetic construct
  source 1..21: mol_type = other DNA; note = TS04/hTS04 CDR-L2 nucleotide sequence
tatagtaccaatcgaccctca

SEQ ID NO: 167 - DNA, 33 bp, synthetic construct
  source 1..33: mol_type = other DNA; note = TS04/hTS04 CDR-L3 nucleotide sequence
ggaagttatgctgcgagtatcgatgagggtatt

SEQ ID NO: 168 - DNA, 33 bp, synthetic construct
  source 1..33: mol_type = other DNA; note = TS05/hTS05 CDR-L1 nucleotide sequence
cagggagacctgctggacgatcaatatacagct

SEQ ID NO: 169 - DNA, 21 bp, synthetic construct
  source 1..21: mol_type = other DNA; note = TS05/hTS05 CDR-L2 nucleotide sequence
aaagacactgagcggccttca

SEQ ID NO: 170 - DNA, 30 bp, synthetic construct
  source 1..30: mol_type = other DNA; note = TS05/hTS05 CDR-L3 nucleotide sequence
ctgtcacttgacagcagcagaatgggtgtt

SEQ ID NO: 171 - DNA, 33 bp, synthetic construct
  source 1..33: mol_type = other DNA; note = TS06/hTS06 CDR-L1 nucleotide sequence
tctggaagcgacttctttagtaatgcagtaggc

SEQ ID NO: 172 - DNA, 21 bp, synthetic construct
  source 1..21: mol_type = other DNA; note = TS06/hTS06 CDR-L2 nucleotide sequence
ggtactacccgtcgaccctca

SEQ ID NO: 173 - DNA, 30 bp, synthetic construct
  source 1..30: mol_type = other DNA; note = TS06/hTS06 CDR-L3 nucleotide sequence
ggaagtactgcccgtagtaactatggtgat

SEQ ID NO: 174 - DNA, 33 bp, synthetic construct; identical to SEQ ID NO: 162
  source 1..33: mol_type = other DNA; note = TS07/hTS07 CDR-L1 nucleotide sequence

SEQ ID NO: 175 - DNA, 21 bp, synthetic construct
  source 1..21: mol_type = other DNA; note = TS07/hTS07 CDR-L2 nucleotide sequence
ggtactactaggcgaccctca

SEQ ID NO: 176 - DNA, 30 bp, synthetic construct
  source 1..30: mol_type = other DNA; note = TS07/hTS07 CDR-L3 nucleotide sequence
ggaggtgctgctggtactaaccatggtgat

SEQ ID NO: 177 - DNA, 30 bp, synthetic construct
  source 1..30: mol_type = other DNA; note = TS08/hTS08 CDR-L1 nucleotide sequence
cagggagacataggaagctcttatgttgcg

SEQ ID NO: 178 - DNA, 21 bp, synthetic construct
  source 1..21: mol_type = other DNA; note = TS08/hTS08 CDR-L2 nucleotide sequence
caaaatagtaagaggccctcg

SEQ ID NO: 179 - DNA, 24 bp, synthetic construct
  source 1..24: mol_type = other DNA; note = TS08/hTS08 CDR-L3 nucleotide sequence
ctgtcagctgacagccgttttgtt

SEQ ID NO: 180 - DNA, 42 bp, synthetic construct
  source 1..42: mol_type = other DNA; note = TS09/hTS09 CDR-L1 nucleotide sequence
tctggaagcagcagcaacatcgggggtggttattatgtgggc

SEQ ID NO: 181 - DNA, 21 bp, synthetic construct
  source 1..21: mol_type = other DNA; note = TS09/hTS09 CDR-L2 nucleotide sequence
caaaacagcaaacgaccgaca

SEQ ID NO: 182 - DNA, 33 bp, synthetic construct
  source 1..33: mol_type = other DNA; note = TS09/hTS09 CDR-L3 nucleotide sequence
tcaacttatgacagcagtattagtgctagtgtt

SEQ ID NO: 183 - DNA, 33 bp, synthetic construct
  source 1..33: mol_type = other DNA; note = TS10/hTS10 CDR-L1 nucleotide sequence
cagggagacgacataggaaggtcttatgttgcg

SEQ ID NO: 184 - DNA, 21 bp, synthetic construct
  source 1..21: mol_type = other DNA; note = TS10/hTS10 CDR-L2 nucleotide sequence
caaaatagtaagaggccctcg

SEQ ID NO: 185 - DNA, 24 bp, synthetic construct
  source 1..24: mol_type = other DNA; note = TS10/hTS10 CDR-L3 nucleotide sequence
ctgtcagctggcagcaggtttgtt

SEQ ID NO: 186 - DNA, 39 bp, synthetic construct
  source 1..39: mol_type = other DNA; note = TS11/hTS11 CDR-L1 nucleotide sequence
tctggaagcagcaggaacgttggtgaatatggtgtaggc

SEQ ID NO: 187 - DNA, 21 bp, synthetic construct
  source 1..21: mol_type = other DNA; note = TS11/hTS11 CDR-L2 nucleotide sequence
ggtactagtagtcgaccctcg

SEQ ID NO: 188 - DNA, 33 bp, synthetic construct
  source 1..33: mol_type = other DNA; note = TS11/hTS11 CDR-L3 nucleotide sequence
gcaactactgacagcagtagaaggaatgttgtt

SEQ ID NO: 189 - DNA, 42 bp, synthetic construct
  source 1..42: mol_type = other DNA; note = TS12/hTS12 CDR-L1 nucleotide sequence
tctggaagcagcagcaacgttggatatggtaattatgtgggc

SEQ ID NO: 190 - DNA, 21 bp, synthetic construct
  source 1..21: mol_type = other DNA; note = TS12/hTS12 CDR-L2 nucleotide sequence
ggtgcaaccaatcgagcctcg

SEQ ID NO: 191 - DNA, 30 bp, synthetic construct
  source 1..30: mol_type = other DNA; note = TS12/hTS12 CDR-L3 nucleotide sequence
gcatcttatgacagcagtagtagaattgtt

SEQ ID NO: 192 - DNA, 39 bp, synthetic construct
  source 1..39: mol_type = other DNA; note = TS13/hTS13 CDR-L1 nucleotide sequence
tctggaagcagcaggaacgttggtgaatatggtgtagct

SEQ ID NO: 193 - DNA, 21 bp, synthetic construct
  source 1..21: mol_type = other DNA; note = TS13/hTS13 CDR-L2 nucleotide sequence
ggtactagcaatcgaccctcg

SEQ ID NO: 194 - DNA, 33 bp, synthetic construct
  source 1..33: mol_type = other DNA; note = TS13/hTS13 CDR-L3 nucleotide sequence
gcagctactgatagcagtaggcgggatgttgtt

SEQ ID NO: 195 - DNA, 42 bp, synthetic construct; identical to SEQ ID NO: 180
  source 1..42: mol_type = other DNA; note = TS14/hTS14 CDR-L1 nucleotide sequence

SEQ ID NO: 196 - DNA, 21 bp, synthetic construct
  source 1..21: mol_type = other DNA; note = TS14/hTS14 CDR-L2 nucleotide sequence
caaaacagcaaacgaccgaca

SEQ ID NO: 197 - DNA, 33 bp, synthetic construct
  source 1..33: mol_type = other DNA; note = TS14/hTS14 CDR-L3 nucleotide sequence
tcaacttatgacagcagtattagtactactgtt

SEQ ID NO: 198 - DNA, 39 bp, synthetic construct; identical to SEQ ID NO: 186
  source 1..39: mol_type = other DNA; note = TS15/hTS15 CDR-L1 nucleotide sequence

SEQ ID NO: 199 - DNA, 21 bp, synthetic construct
  source 1..21: mol_type = other DNA; note = TS15/hTS15 CDR-L2 nucleotide sequence
ggtactcgtagtcgaccctcg

SEQ ID NO: 200 - DNA, 33 bp, synthetic construct; identical to SEQ ID NO: 188
  source 1..33: mol_type = other DNA; note = TS15/hTS15 CDR-L3 nucleotide sequence

SEQ ID NO: 201 - DNA, 42 bp, synthetic construct
  source 1..42: mol_type = other DNA; note = TS16/hTS16 CDR-L1 nucleotide sequence
tcgggaagcagcagcaacgttggatatggtaattatgtgggc

SEQ ID NO: 202 - DNA, 21 bp, synthetic construct
  source 1..21: mol_type = other DNA; note = TS16/hTS16 CDR-L2 nucleotide sequence
ggtgcaaccaatcgagcctcg

SEQ ID NO: 203 - DNA, 30 bp, synthetic construct
  source 1..30: mol_type = other DNA; note = TS16/hTS16 CDR-L3 nucleotide sequence
gcatcttatgacatcaacagtaggattatt

SEQ ID NO: 204 - DNA, 42 bp, synthetic construct
  source 1..42: mol_type = other DNA; note = TS17/hTS17 CDR-L1 nucleotide sequence
tctggaagcagcggcaacgttggatttggtgattatgtggcc

SEQ ID NO: 205 - DNA, 21 bp, synthetic construct
  source 1..21: mol_type = other DNA; note = TS17/hTS17 CDR-L2 nucleotide sequence
cgtgcaacgagtcgagcctcg

SEQ ID NO: 206 - DNA, 30 bp, synthetic construct
  source 1..30: mol_type = other DNA; note = TS17/hTS17 CDR-L3 nucleotide sequence
gcctcttttgacagcagtgccagtggtatt